European Patent Application EP 4 585 617 A1, published July 16, 2025. Title: GIPR ANTIBODY, FUSION PROTEIN THEREOF WITH FGF21, PHARMACEUTICAL COMPOSITION THEREOF, AND USE THEREOF. Applicant: GMAX BIOPHARM LLC. The sequence listing filed with the application follows.

SEQUENCE LISTING (125 sequences)

SEQ ID NO: 1 - protein, 10 aa, synthetic construct
QSVNTDVKSY

SEQ ID NO: 2 - protein, 4 aa, Mus musculus
YASN

SEQ ID NO: 3 - protein, 9 aa, Mus musculus
QHSFDFPYT

SEQ ID NO: 4 - protein, 9 aa, synthetic construct
QHSFDDPYT

SEQ ID NO: 5 - protein, 10 aa, synthetic construct
QSVNTDVYSY

SEQ ID NO: 6 - protein, 10 aa, synthetic construct
QSVNTADYSY

SEQ ID NO: 7 - protein, 10 aa, synthetic construct
QSVNTKDYSY

SEQ ID NO: 8 - protein, 10 aa, synthetic construct
QSVNTDVGSY

SEQ ID NO: 9 - protein, 10 aa, synthetic construct
QSVNTDSYSY

SEQ ID NO: 10 - protein, 10 aa, synthetic construct
QSVNTDVKSY

SEQ ID NO: 11 - protein, 10 aa, synthetic construct
QSVNKDVYSY

SEQ ID NO: 12 - protein, 9 aa, Mus musculus
GYSITSDYA

SEQ ID NO: 13 - protein, 7 aa, Mus musculus
ISYRGIA

SEQ ID NO: 14 - protein, 12 aa, Mus musculus
VRGEYGPGNFDF

SEQ ID NO: 15 - DNA, 30 bp, synthetic construct
  source 1..30: mol_type = other DNA
cagtccgtgaacacagatgtgaagtcttat

SEQ ID NO: 16 - DNA, 12 bp, Mus musculus
  source 1..12: mol_type = other DNA
tatgccagcaac

SEQ ID NO: 17 - DNA, 27 bp, Mus musculus
  source 1..27: mol_type = other DNA
cagcacagcttcgatttcccctacacc

SEQ ID NO: 18 - DNA, 24 bp, synthetic construct
  source 1..24: mol_type = other DNA
cagcacagcttcgatgacccctac

SEQ ID NO: 19 - DNA, 30 bp, synthetic construct
  source 1..30: mol_type = other DNA
cagtccgtgaacacagacgtgtactcttat

SEQ ID NO: 20 - DNA, 30 bp, synthetic construct
  source 1..30: mol_type = other DNA
cagtccgtgaacacagccgactactcttat

SEQ ID NO: 21 - DNA, 30 bp, synthetic construct
  source 1..30: mol_type = other DNA
cagtccgtgaacacaaaggactactcttat

SEQ ID NO: 22 - DNA, 30 bp, synthetic construct
  source 1..30: mol_type = other DNA
cagtccgtgaacacagatgtgggctcttat

SEQ ID NO: 23 - DNA, 30 bp, synthetic construct
  source 1..30: mol_type = other DNA
cagtccgtgaacacagacagctactcttat

SEQ ID NO: 24 - DNA, 30 bp, synthetic construct; identical to SEQ ID NO: 15
  source 1..30: mol_type = other DNA

SEQ ID NO: 25 - DNA, 30 bp, synthetic construct
  source 1..30: mol_type = other DNA
cagtccgtgaacaaggatgtgtactcttat

SEQ ID NO: 26 - DNA, 27 bp, Mus musculus
  source 1..27: mol_type = other DNA
ggctactctatcacaagcgattatgcc

SEQ ID NO: 27 - DNA, 21 bp, Mus musculus
  source 1..21: mol_type = other DNA
atctcctatcgcggcatcgcc

SEQ ID NO: 28 - DNA, 36 bp, Mus musculus
  source 1..36: mol_type = other DNA
gtgcggggcgagtatggccccggcaatttcgacttt

SEQ ID NO: 29 - protein, 111 aa, synthetic construct
DIVLTQSPASLAVSPGQRATITCRASQSVNTDVKSYIHWYQQKPGQPPKLLIYYASNLESGVPARFSGSGSGTDFTLTINPVEANDAANYYCQHSFDFPYTFGGGTKVEIK

SEQ ID NO: 30 - protein, 111 aa, synthetic construct
DIVLTQSPASLAVSPGQRATITCRASQSVNTDVYSYIHWYQQKPGQPPKLLIKYASNLESGVPARFSGSGSGTDFTLTINPVEANDAANYYCQHSFDFPYTFGGGTKVEIK

SEQ ID NO: 31 - protein, 111 aa, synthetic construct
DIVLTQSPASLAVSPGQRATITCRASQSVNTADYSYIHWYQQKPGQPPKLLIKYASNLESGVPARFSGSGSGTDFTLTINPVEANDAANYYCQHSFDFPYTFGGGTKVEIK

SEQ ID NO: 32 - protein, 111 aa, synthetic construct
DIVLTQSPASLAVSPGQRATITCRASQSVNTAVYSYIHWYQQKPGQPPKLLIKYASNLESGVPARFSGSGSGTDFTLTINPVEANDAANYYCQHSFDDPYTFGGGTKVEIK

SEQ ID NO: 33 - protein, 111 aa, synthetic construct
DIVLTQSPASLAVSPGQRATITCRASQSVNTKDYSYIHWYQQKPGQPPKLLIKYASNLESGVPARFSGSGSGTDFTLTINPVEANDAANYYCQHSFDFPYTFGGGTKVEIK

SEQ ID NO: 34 - protein, 111 aa, synthetic construct
DIVLTQSPASLAVSPGQRATITCRASQSVNTDVGSYIHWYQQKPGQPPKLLIKYASNLESGVPARFSGSGSGTDFTLTINPVEANDAANYYCQHSFDFPYTFGGGTKVEIK

SEQ ID NO: 35 - protein, 111 aa, synthetic construct
DIVLTQSPASLAVSPGQRATITCRASQSVNTDSYSYIHWYQQKPGQPPKLLIKYASNLESGVPARFSGSGSGTDFTLTINPVEANDAANYYCQHSFDFPYTFGGGTKVEIK

SEQ ID NO: 36 - protein, 111 aa, synthetic construct
DIVLTQSPASLAVSPGQRATITCRASQSVNTDVKSYIHWYQQKPGQPPKLLIKYASNLESGVPARFSGSGSGTDFTLTINPVEANDAANYYCQHSFDFPYTFGGGTKVEIK

SEQ ID NO: 37 - protein, 111 aa, synthetic construct
DIVLTQSPASLAVSPGQRATITCRASQSVNKDVYSYIHWYQQKPGQPPKLLIKYASNLESGVPARFSGSGSGTDFTLTINPVEANDAANYYCQHSFDFPYTFGGGTKVEIK

SEQ ID NO: 38 - protein, 119 aa, Mus musculus
QVQLQESGPGLVKPSQTLSLTCTVSGYSITSDYAWNWIRQPPGKGVEWMGYISYRGIATYKPSLKSRITISRDTSKNQFSLKLSSVTAADTAVYYCVRGEYGPGNFDFWGQGTTVTVSS

SEQ ID NO: 39 - DNA, 333 bp, synthetic construct
  source 1..333: mol_type = other DNA
gacatcgtgctgacccagtctccagccagcctggccgtgtctccaggacagagggccaccatcacatgcagagccagccagtccgtgaacacagatgtgaagtcttatatccactggtaccagcagaagcctggccagccccctaagctgctgatctattatgccagcaacctggagtccggagtgcctgcacggttctctggaagcggatccggaaccgacttcaccctgacaatcaatccagtggaggccaacgacgccgccaattactattgtcagcacagcttcgatttcccctacacctttggcggcggcacaaaggtggagatcaag

SEQ ID NO: 40 - DNA, 333 bp, synthetic construct
  source 1..333: mol_type = other DNA
gacatcgtgctgacccagtctccagccagcctggccgtgtctccaggacagagggccaccatcacatgcagagccagccagtccgtgaacacagacgtgtactcttatatccactggtaccagcagaagcctggccagccccctaagctgctgatcaagtatgccagcaacctggagtccggagtgcctgcacggttctctggaagcggatccggaaccgacttcaccctgacaatcaatccagtggaggccaacgacgccgccaattactattgtcagcacagcttcgatttcccctacacctttggcggcggcacaaaggtggagatcaag

SEQ ID NO: 41 - DNA, 333 bp, synthetic construct
  source 1..333: mol_type = other DNA
gacatcgtgctgacccagtctccagccagcctggccgtgtctccaggacagagggccaccatcacatgcagagccagccagtccgtgaacacagccgactactcttatatccactggtaccagcagaagcctggccagccccctaagctgctgatcaagtatgccagcaacctggagtccggagtgcctgcacggttctctggaagcggatccggaaccgacttcaccctgacaatcaatccagtggaggccaacgacgccgccaattactattgtcagcacagcttcgatttcccctacacctttggcggcggcacaaaggtggagatcaag

SEQ ID NO: 42 - DNA, 333 bp, synthetic construct
  source 1..333: mol_type = other DNA
gacatcgtgctgacccagtctccagccagcctggccgtgtctccaggacagagggccaccatcacatgcagagccagccagtccgtgaacacagccgtgtactcttatatccactggtaccagcagaagcctggccagccccctaagctgctgatcaagtatgccagcaacctggagtccggagtgcctgcacggttctctggaagcggatccggaaccgacttcaccctgacaatcaatccagtggaggccaacgacgccgccaattactattgtcagcacagcttcgatgacccctacacctttggcggcggcacaaaggtggagatcaag

SEQ ID NO: 43 - DNA, 333 bp, synthetic construct
  source 1..333: mol_type = other DNA
gacatcgtgctgacccagtctccagccagcctggccgtgtctccaggacagagggccaccatcacatgcagagccagccagtccgtgaacacaaaggactactcttatatccactggtaccagcagaagcctggccagccccctaagctgctgatcaagtatgccagcaacctggagtccggagtgcctgcacggttctctggaagcggatccggaaccgacttcaccctgacaatcaatccagtggaggccaacgacgccgccaattactattgtcagcacagcttcgatttcccctacacctttggcggcggcacaaaggtggagatcaag

SEQ ID NO: 44 - DNA, 448 bp, synthetic construct
  source 1..448: mol_type = other DNA
gacatcgtgctgacccagtctccagccagcctggccgtgtctccaggacagagggccaccatcacatgcagagccagccagtccgtgaacacagatgtgggctcttatatccactggtaccagcagaagcctggccagccccctaagctgctgatcaagtatgccagcaacctggagtccggagtgcctgcacggttctctggaagcggatccggaaccgacttcaccctgacaatcaatccagtggaggccaacgacgccgccaattactattgtcagcacagcttcgatttcccctacacctttggcggcggcacaaaggtggagatcaagcgtacggtggctgcaccatctgtcttcatcttcccgccatctgatgagcagttgaaatctggaactgcctctgttgtgtgcctgctgaataacttctatcccagagaggccaaag

SEQ ID NO: 45 - DNA, 333 bp, synthetic construct
  source 1..333: mol_type = other DNA
gacatcgtgctgacccagtctccagccagcctggccgtgtctccaggacagagggccaccatcacatgcagagccagccagtccgtgaacacagacagctactcttatatccactggtaccagcagaagcctggccagccccctaagctgctgatcaagtatgccagcaacctggagtccggagtgcctgcacggttctctggaagcggatccggaaccgacttcaccctgacaatcaatccagtggaggccaacgacgccgccaattactattgtcagcacagcttcgatttcccctacacctttggcggcggcacaaaggtggagatcaag

SEQ ID NO: 46 - DNA, 333 bp, synthetic construct
  source 1..333: mol_type = other DNA
gacatcgtgctgacccagtctccagccagcctggccgtgtctccaggacagagggccaccatcacatgcagagccagccagtccgtgaacacagatgtgaagtcttatatccactggtaccagcagaagcctggccagccccctaagctgctgatcaagtatgccagcaacctggagtccggagtgcctgcacggttctctggaagcggatccggaaccgacttcaccctgacaatcaatccagtggaggccaacgacgccgccaattactattgtcagcacagcttcgatttcccctacacctttggcggcggcacaaaggtggagatcaag

SEQ ID NO: 47 - DNA, 333 bp, synthetic construct
  source 1..333: mol_type = other DNA
gacatcgtgctgacccagtctccagccagcctggccgtgtctccaggacagagggccaccatcacatgcagagccagccagtccgtgaacaaggatgtgtactcttatatccactggtaccagcagaagcctggccagccccctaagctgctgatcaagtatgccagcaacctggagtccggagtgcctgcacggttctctggaagcggatccggaaccgacttcaccctgacaatcaatccagtggaggccaacgacgccgccaattactattgtcagcacagcttcgatttcccctacacctttggcggcggcacaaaggtggagatcaag

SEQ ID NO: 48 - DNA, 357 bp, Mus musculus
  source 1..357: mol_type = other DNA
caggtgcagctgcaggagtccggaccaggactggtgaagccaagccagaccctgtccctgacctgcacagtgtccggctactctatcacaagcgattatgcctggaactggatcaggcagccacctggcaagggagtggagtggatgggctacatctcctatcgcggcatcgccacctacaagccttccctgaagtctcggatcaccatctctagagacacaagcaagaaccagttctctctgaagctgagctccgtgaccgccgccgatacagccgtgtactattgcgtgcggggcgagtatggccccggcaatttcgacttttggggccagggcaccacagtgacagtgtctagc

SEQ ID NO: 49 - protein, 107 aa, Homo sapiens [sequence omitted]

SEQ ID NO: 50 - protein, 326 aa, Homo sapiens
ASTKGPSVFPLAPCSRSTSESTAALGCLVKDYFPEPVTVSWNSGALTSGVHTFPAVLQSSGLYSLSSVVTVPSSNFGTQTYTCNVDHKPSNTKVDKTVERKCCVECPPCPAPPVAGPSVFLFPPKPKDTLMISRTPEVTCVVVDVSHEDPEVQFNWYVDGVEVHNAKTKPREEQFNSTFRVVSVLTVVHQDWLNGKEYKCKVSNKGLPAPIEKTISKTKGQPREPQVYTLPPSREEMTKNQVSLTCLVKGFYPSDIAVEWESNGQPENNYKTTPPMLDSDGSFFLYSKLTVDKSRWQQGNVFSCSVMHEALHNHYTQKSLSLSPGK

SEQ ID NO: 51 - protein, 326 aa, synthetic construct
ASTKGPSVFPLAPCSRSTSESTAALGCLVKDYFPEPVTVSWNSGALTSGVHTFPAVLQSSGLYSLSSVVTVPSSSLGTKTYTCNVDHKPSNTKVDKRVESKYGPPCPPCPAPEAAGGPSVFLFPPKPKDTLMISRTPEVTCVVVDVSQEDPEVQFNWYVDGVEVHNAKTKPREEQFNSTYRVVSVLTVLHQDWLNGKEYKCKVSNKGLPSSIEKTISKAKGQPREPQVYTLPPSQEEMTKNQVSLTCLVKGFYPSDIAVEWESNGQPENNYKTTPPVLDSDGSFFLYSRLTVDKSRWQEGNVFSCSVMHEALHNHYTQKSLSLSLG

SEQ ID NO: 52-60 - skipped (9 entries)

SEQ ID NO: 61 - protein, 5 aa, synthetic construct
GGGGS

SEQ ID NO: 62 - protein, 10 aa, synthetic construct
GGGGSGGGGS

SEQ ID NO: 63 - protein, 15 aa, synthetic construct
GGGGSGGGGSGGGGS

SEQ ID NO: 64 - protein, 20 aa, synthetic construct
GGGGSGGGGSGGGGSGGGGS

SEQ ID NO: 65 - protein, 25 aa, synthetic construct
GGGGSGGGGSGGGGSGGGGSGGGGS

SEQ ID NO: 66 - protein, 30 aa, synthetic construct
GGGGSGGGGSGGGGSGGGGSGGGGSGGGGS

SEQ ID NO: 67 - protein, 35 aa, synthetic construct
GGGGSGGGGSGGGGSGGGGSGGGGSGGGGSGGGGS

SEQ ID NO: 68 - protein, 23 aa, synthetic construct
GSGSATGGSGSGASSGSGSATGS

SEQ ID NO: 69-76 - skipped (8 entries)

SEQ ID NO: 77 - protein, 181 aa, synthetic construct
HPIPDSSPLLQFGGQVRQRYLYTDDAQQTEAHLEIREDGTVGGAADQSPESLLQLKALKPGVIQILGVKTSRFLCQRPDGALYGSLHFDPEACSFRELLLEDGYNVYQSEAHGLPLHCPGNKSPHRDPAPRGPCRFLPLPGLPPALPEPPGILAPQPPDVGSSDPLSMVGPSQGRSPSYAS

SEQ ID NO: 78 - protein, 178 aa, synthetic construct
DSSPLLQFGGQVRQRYLYTDDAQQTEAHLEIREDGTVGGAADQSPESLLQLKALKPGVIQILGVKTSRFLCQRPDGALYGSLHFDPEACSFRERLLEDGYNVYQSEAHGLPLHLPGNKSPHRDPAPRGPARFLPLPGLPPALPEPPGILAPQPPDVGSSDPLSMVTGLEAVRSPSFEK

SEQ ID NO: 79 - protein, 178 aa, synthetic construct
DSSPLLQFGGQVRQAYLYTDDAQQTEAHLEIREDGTVGGAADQSPESLLQLKALKPGVIQILGVKTSRFLCQRPDGALYGSLHFDPEACSFRERLLEDGYNVYQSEAHGLPLHLPGNKSPHRDPAPRGPARFLPLPGLPPALPEPPGILAPQPPDVGSSDPLSMVTGLEAVRSPSFEK

SEQ ID NO: 80 - protein, 178 aa, synthetic construct
DSSPLLQFGGQVRQVYLYTDDAQQTEAHLEIREDGTVGGAADQSPESLLQLKALKPGVIQILGVKTSRFLCQRPDGALYGSLHFDPEACSFRERLLEDGYNVYQSEAHGLPLHLPGNKSPHRDPAPRGPARFLPLPGLPPALPEPPGILAPQPPDVGSSDPLSMVTGLEAVRSPSFEK

SEQ ID NO: 81 - protein, 178 aa, synthetic construct
DSSPLLQFGGQVRQRYLYTDDAQQTEAHLEIREDGTVGGAADQSPESLLQLKALKPGVIQILGVKTSRFLCQRPDGALYGSLHFDPEACSFRERLLEDGYNVYQSEAHGLPLHLPGNKSPHRDPAPRGPAEFLPLPGLPPALPEPPGILAPQPPDVGSSDPLSMVTGLEAVRSPSFEK

SEQ ID NO: 82 - protein, 178 aa, synthetic construct
DSSPLLQFGGQVRQRYLYTDDAQQTEAHLEIREDGTVGGAADQSPESLLQLKALKPGVIQILGVKTSRFLCQRPDGALYGSLHFDPEACSFRERLLEDGYNVYQSEAHGLPLHLPGNKSPHRDPAPRGPAMFLPLPGLPPALPEPPGILAPQPPDVGSSDPLSMVTGLEAVRSPSFEK

SEQ ID NO: 83 - protein, 177 aa, synthetic construct
DSSPLLQFGGQVRQRYLYTDDAQQTEAHLEIREDGTVGGAADQSPESLLQLKALKPGVIQILGVKTSRFLCQRPDGALYGSLHFDPEACSFRERLLEDGYNVYQSEAHGLPLHLPGNKSPHRDPAPRGPARFLPLPGLPPALPEPPGILAPQPPDVGSSDPLSMVTGLEARSPSFEK

SEQ ID NO: 84 - protein, 177 aa, synthetic construct
DSSPLLQFGGQVRQRYLYTDDAQQTEAHLEIREDGTVGGAADQSPESLLQLKALKPGVIQILGVKTSRFLCQRPDGALYGSLHFDPEACSFRERLLEDGYNVYQSEAHGLPLHLPGNKSPHRDPAPRGPARFLPLPGLPPALPEPPGILAPQPPDVGSSDPLSMVTGLEARSPSFES

SEQ ID NO: 85 - protein, 177 aa, synthetic construct
DSSPLLQFGGQVRQRYLYTDDAQQTEAHLEIREDGTVGGAADQSPESLLQLKALKPGVIQILGVKTSRFLCQRPDGALYGSLHFDPEACSFRERLLEDGYNVYQSEAHGLPLHLPGNKSPHRDPAPRGPARFLPLPGLPPALPEPPGILAPQPPDVGSSDPLSMVTGLEAKSPSFQK

SEQ ID NO: 86 - protein, 177 aa, synthetic construct
DSSPLLQFGGQVRQRYLYTDDAQQTEAHLEIREDGTVGGAADQSPESLLQLKALKPGVIQILGVKTSRFLCQRPDGALYGSLHFDPEACSFRERLLEDGYNVYQSEAHGLPLHLPGNKSPHRDPAPRGPARFLPLPGLPPALPEPPGILAPQPPDVGSSDPLSMVTGLEARSPSFDK

SEQ ID NO: 87 - protein, 177 aa, synthetic construct
DSSPLLQFGGQVRQRYLYTDDAQQTEAHLEIREDGTVGGAADQSPESLLQLKALKPGVIQILGVKTSRFLCQRPDGALYGSLHFDPEACSFRERLLEDGYNVYQSEAHGLPLHLPGNKSPHRDPAPRGPARFLPLPGLPPALPEPPGILAPQPPDVGSSDPLSMVTGLEARSPSFQK

SEQ ID NO: 88 - protein, 178 aa, synthetic construct
DSSPLLQFGGQVRQAYLYTDDAQQTEAHLEIREDGTVGGAADQSPESLLQLKALKPGVIQILGVKTSRFLCQRPDGALYGSLHFDPEACSFRERLLEDGYNVYQSEAHGLPLHCPGNKSPHRDPAPRGPCRFLPLPGLPPALPEPPGILAPQPPDVGSSDPLSMVTGLEAVRSPSFEK

SEQ ID NO: 89 - protein, 182 aa, synthetic construct
HPIPDSSPLLQFGGQVRQAYLYTDDAQQTEAHLEIREDGTVGGAADQSPESLLQLKALKPGVIQILGVKTSRFLCQRPDGALYGSLHFDPEACSFRERLLEDGYNVYQSEAHGLPLHLPGNKSPHRDPAPRGPARFLPLPGLPPALPEPPGILAPQPPDVGSSDPLSMVTGLEAVRSPSFEK

SEQ ID NO: 90-102 - skipped (13 entries)

SEQ ID NO: 103 - protein, 218 aa, synthetic construct
DIVLTQSPASLAVSPGQRATITCRASQSVNTDVKSYIHWYQQKPGQPPKLLIYYASNLESGVPARFSGSGSGTDFTLTINPVEANDAANYYCQHSFDFPYTFGGGTKVEIKRTVAAPSVFIFPPSDEQLKSGTASVVCLLNNFYPREAKVQWKVDNALQSGNSQESVTEQDSKDSTYSLSSTLTLSKADYEKHKVYACEVTHQGLSSPVTKSFNRGEC

SEQ ID NO: 104 - protein, 650 aa, synthetic construct
QVQLQESGPGLVKPSQTLSLTCTVSGYSITSDYAWNWIRQPPGKGVEWMGYISYRGIATYKPSLKSRITISRDTSKNQFSLKLSSVTAADTAVYYCVRGEYGPGNFDFWGQGTTVTVSSASTKGPSVFPLAPCSRSTSESTAALGCLVKDYFPEPVTVSWNSGALTSGVHTFPAVLQSSGLYSLSSVVTVPSSNFGTQTYTCNVDHKPSNTKVDKTVERKCCVECPPCPAPPVAGPSVFLFPPKPKDTLMISRTPEVTCVVVDVSHEDPEVQFNWYVDGVEVHNAKTKPREEQFNSTFRVVSVLTVVHQDWLNGKEYKCKVSNKGLPAPIEKTISKTKGQPREPQVYTLPPSREEMTKNQVSLTCLVKGFYPSDIAVEWESNGQPENNYKTTPPMLDSDGSFFLYSKLTVDKSRWQQGNVFSCSVMHEALHNHYTQKSLSLSPGKGSGSATGGSGSGASSGSGSATGSHPIPDSSPLLQFGGQVRQAYLYTDDAQQTEAHLEIREDGTVGGAADQSPESLLQLKALKPGVIQILGVKTSRFLCQRPDGALYGSLHFDPEACSFRERLLEDGYNVYQSEAHGLPLHLPGNKSPHRDPAPRGPARFLPLPGLPPALPEPPGILAPQPPDVGSSDPLSMVTGLEAVRSPSFEK

SEQ ID NO: 105 - protein, 650 aa, synthetic construct
QVQLQESGPGLVKPSQTLSLTCTVSGYSITSDYAWNWIRQPPGKGVEWMGYISYRGIATYKPSLKSRITISRDTSKNQFSLKLSSVTAADTAVYYCVRGEYGPGNFDFWGQGTTVTVSSASTKGPSVFPLAPCSRSTSESTAALGCLVKDYFPEPVTVSWNSGALTSGVHTFPAVLQSSGLYSLSSVVTVPSSSLGTKTYTCNVDHKPSNTKVDKRVESKYGPPCPPCPAPEAAGGPSVFLFPPKPKDTLMISRTPEVTCVVVDVSQEDPEVQFNWYVDGVEVHNAKTKPREEQFNSTYRVVSVLTVLHQDWLNGKEYKCKVSNKGLPSSIEKTISKAKGQPREPQVYTLPPSQEEMTKNQVSLTCLVKGFYPSDIAVEWESNGQPENNYKTTPPVLDSDGSFFLYSRLTVDKSRWQEGNVFSCSVMHEALHNHYTQKSLSLSLGGSGSATGGSGSGASSGSGSATGSHPIPDSSPLLQFGGQVRQAYLYTDDAQQTEAHLEIREDGTVGGAADQSPESLLQLKALKPGVIQILGVKTSRFLCQRPDGALYGSLHFDPEACSFRERLLEDGYNVYQSEAHGLPLHLPGNKSPHRDPAPRGPARFLPLPGLPPALPEPPGILAPQPPDVGSSDPLSMVTGLEAVRSPSFEK

SEQ ID NO: 106 - protein, 642 aa, synthetic construct
QVQLQESGPGLVKPSQTLSLTCTVSGYSITSDYAWNWIRQPPGKGVEWMGYISYRGIATYKPSLKSRITISRDTSKNQFSLKLSSVTAADTAVYYCVRGEYGPGNFDFWGQGTTVTVSSASTKGPSVFPLAPCSRSTSESTAALGCLVKDYFPEPVTVSWNSGALTSGVHTFPAVLQSSGLYSLSSVVTVPSSNFGTQTYTCNVDHKPSNTKVDKTVERKCCVECPPCPAPPVAGPSVFLFPPKPKDTLMISRTPEVTCVVVDVSHEDPEVQFNWYVDGVEVHNAKTKPREEQFNSTFRVVSVLTVVHQDWLNGKEYKCKVSNKGLPAPIEKTISKTKGQPREPQVYTLPPSREEMTKNQVSLTCLVKGFYPSDIAVEWESNGQPENNYKTTPPMLDSDGSFFLYSKLTVDKSRWQQGNVFSCSVMHEALHNHYTQKSLSLSPGKGGGGSGGGGSGGGGSHPIPDSSPLLQFGGQVRQAYLYTDDAQQTEAHLEIREDGTVGGAADQSPESLLQLKALKPGVIQILGVKTSRFLCQRPDGALYGSLHFDPEACSFRERLLEDGYNVYQSEAHGLPLHLPGNKSPHRDPAPRGPARFLPLPGLPPALPEPPGILAPQPPDVGSSDPLSMVTGLEAVRSPSFEK

SEQ ID NO: 107-110 - skipped (4 entries)

SEQ ID NO: 111 - protein, 445 aa, synthetic construct
QVQLQESGPGLVKPSQTLSLTCTVSGYSITSDYAWNWIRQPPGKGVEWMGYISYRGIATYKPSLKSRITISRDTSKNQFSLKLSSVTAADTAVYYCVRGEYGPGNFDFWGQGTTVTVSSASTKGPSVFPLAPCSRSTSESTAALGCLVKDYFPEPVTVSWNSGALTSGVHTFPAVLQSSGLYSLSSVVTVPSSNFGTQTYTCNVDHKPSNTKVDKTVERKCCVECPPCPAPPVAGPSVFLFPPKPKDTLMISRTPEVTCVVVDVSHEDPEVQFNWYVDGVEVHNAKTKPREEQFNSTFRVVSVLTVVHQDWLNGKEYKCKVSNKGLPAPIEKTISKTKGQPREPQVYTLPPSREEMTKNQVSLTCLVKGFYPSDIAVEWESNGQPENNYKTTPPMLDSDGSFFLYSKLTVDKSRWQQGNVFSCSVMHEALHNHYTQKSLSLSPGK

SEQ ID NO: 112 - protein, 445 aa, synthetic construct
QVQLQESGPGLVKPSQTLSLTCTVSGYSITSDYAWNWIRQPPGKGVEWMGYISYRGIATYKPSLKSRITISRDTSKNQFSLKLSSVTAADTAVYYCVRGEYGPGNFDFWGQGTTVTVSSASTKGPSVFPLAPCSRSTSESTAALGCLVKDYFPEPVTVSWNSGALTSGVHTFPAVLQSSGLYSLSSVVTVPSSSLGTKTYTCNVDHKPSNTKVDKRVESKYGPPCPPCPAPEAAGGPSVFLFPPKPKDTLMISRTPEVTCVVVDVSQEDPEVQFNWYVDGVEVHNAKTKPREEQFNSTYRVVSVLTVLHQDWLNGKEYKCKVSNKGLPSSIEKTISKAKGQPREPQVYTLPPSQEEMTKNQVSLTCLVKGFYPSDIAVEWESNGQPENNYKTTPPVLDSDGSFFLYSRLTVDKSRWQEGNVFSCSVMHEALHNHYTQKSLSLSLG

SEQ ID NO: 113 - DNA, 1335 bp, synthetic construct
  source 1..1335: mol_type = other DNA
caggtgcagctgcaggagtccggaccaggactggtgaagccaagccagaccctgtccctgacctgcacagtgtccggctactctatcacaagcgattatgcctggaactggatcaggcagccacctggcaagggagtggagtggatgggctacatctcctatcgcggcatcgccacctacaagccttccctgaagtctcggatcaccatctctagagacacaagcaagaaccagttctctctgaagctgagctccgtgaccgccgccgatacagccgtgtactattgcgtgcggggcgagtatggccccggcaatttcgacttttggggccagggcaccacagtgacagtgtctagcgcgtcgaccaagggcccatcggtcttccccctggcgccctgctccaggagcacctccgagagcacagcggccctgggctgcctggtcaaggactacttccccgaaccggtgacggtgtcgtggaactcaggcgctctgaccagcggcgtgcacaccttcccagctgtcctacagtcctcaggactctactccctcagcagcgtggtgaccgtgccctccagcaacttcggcacccagacctacacctgcaacgtagatcacaagcccagcaacaccaaggtggacaagacagttgagcgcaaatgttgtgtcgagtgcccaccgtgcccagcaccacctgtggcaggaccgtcagtcttcctcttccccccaaaacccaaggacaccctcatgatctcccggacccctgaggtcacgtgcgtggtggtggacgtgagccacgaagaccccgaggtccagttcaactggtacgtggacggcgtggaggtgcataatgccaagacaaagccacgggaggagcagttcaacagcacgttccgtgtggtcagcgtcctcaccgttgtgcaccaggactggctgaacggcaaggagtacaagtgcaaggtctccaacaaaggcctcccagcccccatcgagaaaaccatctccaaaaccaaagggcagccccgagaaccacaggtgtacaccctgcccccatcccgggaggagatgaccaagaaccaggtcagcctgacctgcctggtcaaaggcttctaccccagcgacatcgccgtggagtgggagagcaatgggcagccggagaacaactacaagaccacacctcccatgctggactccgacggctccttcttcctctacagcaagctcaccgtggacaagagcaggtggcagcaggggaacgtcttctcatgctccgtgatgcatgaggctctgcacaaccactacacgcagaagagcctctccctgtctccgggtaaa

SEQ ID NO: 114 - DNA, 1335 bp, synthetic construct
  source 1..1335: mol_type = other DNA
caggtgcagctgcaggagtccggaccaggactggtgaagccaagccagaccctgtccctgacctgcacagtgtccggctactctatcacaagcgattatgcctggaactggatcaggcagccacctggcaagggagtggagtggatgggctacatctcctatcgcggcatcgccacctacaagccttccctgaagtctcggatcaccatctctagagacacaagcaagaaccagttctctctgaagctgagctccgtgaccgccgccgatacagccgtgtactattgcgtgcggggcgagtatggccccggcaatttcgacttttggggccagggcaccacagtgacagtgtctagcgcgtcgaccaagggcccatcggtcttccccctggcgccctgctccaggagcacctccgagagcacagcggccctgggctgcctggtcaaggactacttccccgaaccggtgacggtgtcgtggaactcaggcgctctgaccagcggcgtgcacaccttcccagctgtcctacagtcctcaggactctactccctcagcagcgtggtgaccgtgccctccagcagcctcggcaccaagacctacacctgcaacgtagatcacaagcccagcaacaccaaggtggacaagcgggttgagtccaaatatggtcccccatgcccaccctgcccagcacctgaggccgccgggggaccatcagtcttcctgttccccccaaaacccaaggacactctcatgatctcccggacccctgaggtcacgtgcgtggtggtggacgtgagccaggaagaccccgaggtccagttcaactggtacgtggatggcgtggaggtgcataatgccaagacaaagccgcgggaggagcagttcaacagcacgtaccgtgtggtcagcgtcctcaccgtcctgcaccaggactggctgaacggcaaggagtacaagtgcaaggtctccaacaaaggcctcccgtcctccatcgagaaaaccatctccaaagccaaagggcagccccgagagccacaggtgtacaccctgcccccatcccaggaggagatgaccaagaaccaggtcagcctgacctgcctggtcaaaggcttctaccccagcgacatcgccgtggagtgggaaagcaatgggcagccggagaacaactacaagaccacgcctcccgtgctggactccgacggctccttcttcctctacagcaggctaaccgtggacaagagcaggtggcaggaggggaatgtcttctcatgctccgtgatgcatgaggctctgcacaaccactacacacagaagagcctctccctgtctctgggt

SEQ ID NO: 115 - protein, 178 aa, synthetic construct; identical to SEQ ID NO: 79

SEQ ID NO: 116 - protein, 182 aa, synthetic construct
HPIPDSSPLLQFGGQVRQAYLYTDDAQQTEAHLEIREDGTVGGAADQSPESLLQLKALKPGVIQILGVKTSRFLCQRPDGALYGSLHFDPEACSFRERLLEDGYNVYQSEAHGLPLHLPGNESPHRDPAPRGPARFLPLPGLPPALPEPPGILAPQPPDVGSSDPLSMVTGLEAVRSPSFEK

SEQ ID NO: 117 - protein, 182 aa, synthetic construct
HPIPDSSPLLQFGGQVRQAYLYTDDAQQTEAHLEIREDGTVGGAADQSPESLLQLKALKPGVIQILGVKTSRFLCQRPDGALYGSLHFDPEACSFRERLLEDGYNVYQSEAHGLPLHLPGNKSPHRDPAPRGPNRFLPLPGLPPALPEPPGILAPQPPDVGSSDPLSMVTGLEAVRSPSFEK

SEQ ID NO: 118 - protein, 178 aa, synthetic construct
DSSPLLQFGGQVRQAYLYTDDAQQTEAHLEIREDGTVGGAADQSPESLLQLKALKPGVIQILGVKTSRFLCQRPDGALYGSLHFDPEACSFRERLLEDGYNVYQSEAHGLPLHLPGNESPHRDPAPRGPNRFLPLPGLPPALPEPPGILAPQPPDVGSSDPLSMVTGLEAVRSPSFEK

SEQ ID NO: 119 - protein, 650 aa, synthetic construct
  VARIANT 469..472: note = These 4 residues are HPIP or non-existent
  VARIANT 487: note = This residue is R or A
  VARIANT 566: note = This residue is L or R
  VARIANT 590: note = This residue is K or E
  VARIANT 602: note = This residue is A or N
QVQLQESGPGLVKPSQTLSLTCTVSGYSITSDYAWNWIRQPPGKGVEWMGYISYRGIATYKPSLKSRITISRDTSKNQFSLKLSSVTAADTAVYYCVRGEYGPGNFDFWGQGTTVTVSSASTKGPSVFPLAPCSRSTSESTAALGCLVKDYFPEPVTVSWNSGALTSGVHTFPAVLQSSGLYSLSSVVTVPSSNFGTQTYTCNVDHKPSNTKVDKTVERKCCVECPPCPAPPVAGPSVFLFPPKPKDTLMISRTPEVTCVVVDVSHEDPEVQFNWYVDGVEVHNAKTKPREEQFNSTFRVVSVLTVVHQDWLNGKEYKCKVSNKGLPAPIEKTISKTKGQPREPQVYTLPPSREEMTKNQVSLTCLVKGFYPSDIAVEWESNGQPENNYKTTPPMLDSDGSFFLYSKLTVDKSRWQQGNVFSCSVMHEALHNHYTQKSLSLSPGKGSGSATGGSGSGASSGSGSATGSXXXXDSSPLLQFGGQVRQXYLYTDDAQQTEAHLEIREDGTVGGAADQSPESLLQLKALKPGVIQILGVKTSRFLCQRPDGALYGSLHFDPEACSFREXLLEDGYNVYQSEAHGLPLHLPGNXSPHRDPAPRGPXRFLPLPGLPPALPEPPGILAPQPPDVGSSDPLSMVTGLEAVRSPSFEK

SEQ ID NO: 120 - protein, 650 aa, synthetic construct
  VARIANT 469..472: note = There 4 residues are HPIP or non-existent
  VARIANT 487: note = This residue is R or A
  VARIANT 566: note = This residue is L or R
  VARIANT 590: note = This residue is K or E
  VARIANT 602: note = This residue is A or N
QVQLQESGPGLVKPSQTLSLTCTVSGYSITSDYAWNWIRQPPGKGVEWMGYISYRGIATYKPSLKSRITISRDTSKNQFSLKLSSVTAADTAVYYCVRGEYGPGNFDFWGQGTTVTVSSASTKGPSVFPLAPCSRSTSESTAALGCLVKDYFPEPVTVSWNSGALTSGVHTFPAVLQSSGLYSLSSVVTVPSSSLGTKTYTCNVDHKPSNTKVDKRVESKYGPPCPPCPAPEAAGGPSVFLFPPKPKDTLMISRTPEVTCVVVDVSQEDPEVQFNWYVDGVEVHNAKTKPREEQFNSTYRVVSVLTVLHQDWLNGKEYKCKVSNKGLPSSIEKTISKAKGQPREPQVYTLPPSQEEMTKNQVSLTCLVKGFYPSDIAVEWESNGQPENNYKTTPPVLDSDGSFFLYSRLTVDKSRWQEGNVFSCSVMHEALHNHYTQKSLSLSLGGSGSATGGSGSGASSGSGSATGSXXXXDSSPLLQFGGQVRQXYLYTDDAQQTEAHLEIREDGTVGGAADQSPESLLQLKALKPGVIQILGVKTSRFLCQRPDGALYGSLHFDPEACSFREXLLEDGYNVYQSEAHGLPLHLPGNXSPHRDPAPRGPXRFLPLPGLPPALPEPPGILAPQPPDVGSSDPLSMVTGLEAVRSPSFEK

SEQ ID NO: 121 - protein, 642 aa, synthetic construct
  VARIANT 461..464: note = There 4 residues are HPIP or non-existent
  VARIANT 479: note = This residue is R or A
  VARIANT 558: note = This residue is L or R
  VARIANT 582: note = This residue is K or E
  VARIANT 594: note = This residue is A or N
QVQLQESGPGLVKPSQTLSLTCTVSGYSITSDYAWNWIRQPPGKGVEWMGYISYRGIATYKPSLKSRITISRDTSKNQFSLKLSSVTAADTAVYYCVRGEYGPGNFDFWGQGTTVTVSSASTKGPSVFPLAPCSRSTSESTAALGCLVKDYFPEPVTVSWNSGALTSGVHTFPAVLQSSGLYSLSSVVTVPSSNFGTQTYTCNVDHKPSNTKVDKTVERKCCVECPPCPAPPVAGPSVFLFPPKPKDTLMISRTPEVTCVVVDVSHEDPEVQFNWYVDGVEVHNAKTKPREEQFNSTFRVVSVLTVVHQDWLNGKEYKCKVSNKGLPAPIEKTISKTKGQPREPQVYTLPPSREEMTKNQVSLTCLVKGFYPSDIAVEWESNGQPENNYKTTPPMLDSDGSFFLYSKLTVDKSRWQQGNVFSCSVMHEALHNHYTQKSLSLSPGKGGGGSGGGGSGGGGSXXXXDSSPLLQFGGQVRQXYLYTDDAQQTEAHLEIREDGTVGGAADQSPESLLQLKALKPGVIQILGVKTSRFLCQRPDGALYGSLHFDPEACSFREXLLEDGYNVYQSEAHGLPLHLPGNXSPHRDPAPRGPXRFLPLPGLPPALPEPPGILAPQPPDVGSSDPLSMVTGLEAVRSPSFEK

SEQ ID NO: 122 - protein, 182 aa, synthetic construct
  VARIANT 1..4: note = These 4 residues are HPIP or non-existent
  VARIANT 19: note = This residue is R or A
  VARIANT 98: note = This residue is L or R
  VARIANT 122: note = This residue is K or E
  VARIANT 134: note = This residue is A or N
XXXXDSSPLLQFGGQVRQXYLYTDDAQQTEAHLEIREDGTVGGAADQSPESLLQLKALKPGVIQILGVKTSRFLCQRPDGALYGSLHFDPEACSFREXLLEDGYNVYQSEAHGLPLHLPGNXSPHRDPAPRGPXRFLPLPGLPPALPEPPGILAPQPPDVGSSDPLSMVTGLEAVRSPSFEK

SEQ ID NO: 123 - protein, 646 aa, synthetic construct
QVQLQESGPGLVKPSQTLSLTCTVSGYSITSDYAWNWIRQPPGKGVEWMGYISYRGIATYKPSLKSRITISRDTSKNQFSLKLSSVTAADTAVYYCVRGEYGPGNFDFWGQGTTVTVSSASTKGPSVFPLAPCSRSTSESTAALGCLVKDYFPEPVTVSWNSGALTSGVHTFPAVLQSSGLYSLSSVVTVPSSNFGTQTYTCNVDHKPSNTKVDKTVERKCCVECPPCPAPPVAGPSVFLFPPKPKDTLMISRTPEVTCVVVDVSHEDPEVQFNWYVDGVEVHNAKTKPREEQFNSTFRVVSVLTVVHQDWLNGKEYKCKVSNKGLPAPIEKTISKTKGQPREPQVYTLPPSREEMTKNQVSLTCLVKGFYPSDIAVEWESNGQPENNYKTTPPMLDSDGSFFLYSKLTVDKSRWQQGNVFSCSVMHEALHNHYTQKSLSLSPGKGSGSATGGSGSGASSGSGSATGSDSSPLLQFGGQVRQAYLYTDDAQQTEAHLEIREDGTVGGAADQSPESLLQLKALKPGVIQILGVKTSRFLCQRPDGALYGSLHFDPEACSFRERLLEDGYNVYQSEAHGLPLHLPGNESPHRDPAPRGPNRFLPLPGLPPALPEPPGILAPQPPDVGSSDPLSMVTGLEAVRSPSFEK

SEQ ID NO: 124 - protein, 646 aa, synthetic construct
QVQLQESGPGLVKPSQTLSLTCTVSGYSITSDYAWNWIRQPPGKGVEWMGYISYRGIATYKPSLKSRITISRDTSKNQFSLKLSSVTAADTAVYYCVRGEYGPGNFDFWGQGTTVTVSSASTKGPSVFPLAPCSRSTSESTAALGCLVKDYFPEPVTVSWNSGALTSGVHTFPAVLQSSGLYSLSSVVTVPSSSLGTKTYTCNVDHKPSNTKVDKRVESKYGPPCPPCPAPEAAGGPSVFLFPPKPKDTLMISRTPEVTCVVVDVSQEDPEVQFNWYVDGVEVHNAKTKPREEQFNSTYRVVSVLTVLHQDWLNGKEYKCKVSNKGLPSSIEKTISKAKGQPREPQVYTLPPSQEEMTKNQVSLTCLVKGFYPSDIAVEWESNGQPENNYKTTPPVLDSDGSFFLYSRLTVDKSRWQEGNVFSCSVMHEALHNHYTQKSLSLSLGGSGSATGGSGSGASSGSGSATGSDSSPLLQFGGQVRQAYLYTDDAQQTEAHLEIREDGTVGGAADQSPESLLQLKALKPGVIQILGVKTSRFLCQRPDGALYGSLHFDPEACSFRERLLEDGYNVYQSEAHGLPLHLPGNESPHRDPAPRGPNRFLPLPGLPPALPEPPGILAPQPPDVGSSDPLSMVTGLEAVRSPSFEK

SEQ ID NO: 125 - protein, 638 aa, synthetic construct
QVQLQESGPGLVKPSQTLSLTCTVSGYSITSDYAWNWIRQPPGKGVEWMGYISYRGIATYKPSLKSRITISRDTSKNQFSLKLSSVTAADTAVYYCVRGEYGPGNFDFWGQGTTVTVSSASTKGPSVFPLAPCSRSTSESTAALGCLVKDYFPEPVTVSWNSGALTSGVHTFPAVLQSSGLYSLSSVVTVPSSNFGTQTYTCNVDHKPSNTKVDKTVERKCCVECPPCPAPPVAGPSVFLFPPKPKDTLMISRTPEVTCVVVDVSHEDPEVQFNWYVDGVEVHNAKTKPREEQFNSTFRVVSVLTVVHQDWLNGKEYKCKVSNKGLPAPIEKTISKTKGQPREPQVYTLPPSREEMTKNQVSLTCLVKGFYPSDIAVEWESNGQPENNYKTTPPMLDSDGSFFLYSKLTVDKSRWQQGNVFSCSVMHEALHNHYTQKSLSLSPGKGGGGSGGGGSGGGGSDSSPLLQFGGQVRQAYLYTDDAQQTEAHLEIREDGTVGGAADQSPESLLQLKALKPGVIQILGVKTSRFLCQRPDGALYGSLHFDPEACSFRERLLEDGYNVYQSEAHGLPLHLPGNESPHRDPAPRGPNRFLPLPGLPPALPEPPGILAPQPPDVGSSDPLSMVTGLEAVRSPSFEK